European Patent Specification EP 2 814 967 B1, published June 3, 2026. Title: Improving drought resistance in plants: UPL3. Applicant: Keygene N.V. The sequence listing filed with the application follows.

SEQUENCE LISTING (10 sequences)

SEQ ID NO: 1 - DNA, 5667 bp, Arabidopsis thaliana
atggaaactcggagccgcaagcgggcggaggcgacctcagctgccccatcttcttcttcttcttctcctcctcctcctccctctgcctctggtcccaccacccgcagcaaacgcgctcgtctttcttcttcttcttcttcctcacttgcccccactcctccttcttcctccaccaccacccgctctcgttcttctcgctctgccgccgccgctgctcccatggacacctccaccgactcttctggatttcgccgaggcggacgtggtaacaggggaaacaacaacgataattctgacaaaggtaaggagaaggaacatgacgttaggattagggagcgtgaaagagaaagagaccgagccagagaacaactcaacatggatgctgccgccgccgctgctaggagcgctgacgaggatgacgacaatgacagtgaggatggcaacggcggtttcatgcatcctaacatgagctctgcgagcagtgctttacaaggcttgctcaggaagctcggtgctggattggatgacttgcttccttcttccggtatcggctctgcttcttcctcccacttgaatggaaggatgaagaagattctctctggcttgcgcgctgaaggagaagagggaaaacaggtcgaggctttaacccagctttgtgagatgttatccattgggaccgaagactcgcttagcaccttctctgttgattccttcgtcccagttcttgtcggtctacttaaccatgaaagcaatcccgacattatgcttcttgctgccagggctcttacccatctatgtgatgtcttgccgtcttcttgtgctgctgttgtacattacggggcagtttcatgcttggtggccagattgctaaccatagaatacatggacttggcggaacagtctctgcaagctctcaaaaagatatctcaggagcacccaactgcctgtttgcgagctggtgctcttatggctgtgctctcgtatctggatttcttctccactggtgttcagcgcgtagcactatctactgctgccaacatgtgcaagaaactaccttctgatgcatctgattatgttatggaagctgtacctttgctgacaaacctacttcagtatcatgattcgaaggttttggaatatgcttctatctgtctgactcgaattgctgaagcatttgcaccgtatcccgagaaattagatgaattatgtaaccatggcctggtgacgcaagctgcgtctcttatttccacgagcaattcaggaggtgggcaagcatctcttagtgtgtcaacatacacggggttaatccgattactttctacctgtgcgagcgggtcacctcttggattcaggacattacttcttcttggtattagtagcattcttaaggatattctgttgggttctggggtctctgctaatgcatctgtatccccagcactgagccggcctgcagatcagatttatgagatagtcaacctagcgaatgagctcctccctccattgccagaaggagttatctctcttcctactagcacaaacgctcttgtgaaaggttcatgccaaaagaaatctagtccaagtacttcaggaaaacaagaagatattctaaaaatttcaccaagagaaaaattacttggtgatcaacctgaacttctgcagcagtttggattggatcttcttccagttttagtgcagatctatggttctagtgtcaatggtacgattcgccataaatgtctctcagtcattggaaagttgatgtatttcagcagttcagaaatgattcaatctctaattggtgacacaaatatttcgagcttcttggctggtgtcttggcatggaaagacccacaggtcttggttcctgctctacaagttgcagagattttgatggaaaagcttcctgaaacattctcgaaagtgtttgtgagggaaggggtagtccatgctgtagatcaacttgtcttggttggtaaaccatcccatgcctcacctactgataaggacaatgactgtgtacccggatctgcacgatctaggcgttatagacggcgcagtagtaatgccaattccgatggaaaccagtcggaagagcctaagaatcctgcgtcccttaccataggggcaaaccataattcccttgatactcctacagctagcttcatgctaagggaaacagttagttcctgcgccaaagcattcaaagacaagtacttcccgtctgatggtggggatgttgatgttggagttacagatgatcttttacatctgaagaatctttgcacgaagctaactgctggtatagatgatcataaagtgaaaggaaagggaaaatctaaagcctctgggccattccttggcgatttctctgctagcaaggaagagtacttgattggtgtcatttctgagatacttggcgagataagtaaaggggatggtgtctcaacttttgagtttattggcagtggtgtggttgcagcattgcttaactatttttcttgtggatacttttccaaagagaagatctccgaacttaatttgcccaaacttcgccaggagggactcagaaggtttaaagcttttctagaagtcgctcttccttttgatggtaatgagggaaaggtccctcctatgacagttttgattcagaaacttcaaaatgctttatcgtcactggagcgctttcctgttgtccttagccatccctcaaggtcactaagtggaagtgctcggctctcctcgggtttgagtgctttggcacatcctttaaagttgcgattatgccgagcatctggagagaaaacactacgtgattactcctccaatattgtacttatagatccattggcaagcttagcagcagtggaggaatttctgtggccccgagttcaacggagtgaatctgctctgaagccggcagcgcctattggcaatacagagccaggcacgttacctagcggtgctggtgtttcatcaccatcttcgtcaactccagcttcaaccactcgtcgtcattcttctagatctcgatcggcaattaacatcggtgatacttcaaagaaagatcctgtgcatgagaaaggtaccagctcatcgaaaggaaaaggtaaaggcgttatgaaaccggctcaggcggataaggggcctcaaacaaggagcaatgctcaaaagagagctgttcttgacaaagatactcaaatgaaaccagctagcggagactccagttctgaggatgaggaattggaaatatccccagtcgacattgatgatgccttggtgattgaagaggatgacatttctgatgatgaagatgatgataatgaagatgttttggatgacagtcttcccatgtgcacgcctgataaagtccatgatgtgaaattggcggactcagtggatgatgatggtctagcaaccagcggccgacaaatgaatccagcttctggaggcactagtggagccgcagcagcaagggcatctgattctattgatactggcattgggaattcctatggttctagaggtgcactctcctttgctgctgcagcgatggctgggcttggagctgccagtggtagaggtatcaggggaagtagggacttgcatggacgtaccctaaatcgaagttcagatgagccctctaagttgatatttactgcggcaggaaaacaacttagtaggcatttgacgatttatcaggctgtacagcgacaacttatgctagatgaagatgatgatgacaggtttggtggcagtgatctagtctcaagtgatggaagcagattcaatgatatttacaccatcatgtaccagaggccagacagccaagtgaataggttgtctgttggtggagcaagttctaccacaccgtcaaaatccacgaaatctgctactaccaattccagtgtagaatctcagtcacatagggcatctcttttggatagtatcttacaaggggagcttccatgcgaccttgagaagtcgaattctacatataatgttctggcactgttacgtgtattagagggtttaaatcagctttgccctcgtttaagagcccaaactctttccgatcgttttgcagagggtaaaattacaagtctagatgatctgagtacaactgctgctaaggttcctcttgatgaatttgtcaatagcaaacttacacccaaattggctcgacaaatccaggatgcgcttgctttgtgcagtggaagtcttccctcttggtgctaccagttgactagagcatgcccatttttgtttccgtttcaaacccggagacagtatttctactcgactgcttttgggttgtctcgtgcattgaatcgtttgcagcagcagcaaggtgctgacggcagtgggtctacaaatgaacgagagatgagaatagggagattgcagcgccagaaagtccgtgtatcccgaaataggatattagattctgctgcaaaagttatggagatgtattctagccagaaagctgtgcttgaagtagaatattttggtgaagttggtactggtctaggccctacccttgagttttacacacttctaagccatgatctgcaaaaggcttccctagggatgtggagatcaagttctggtgacaaggtatctatgcaaattggtagagatgagattgaagacggaaaaccatctgcagctaacagagatatagttctggcaccacttggattgtttcctcggccttggccctcaacagctgacatatctgaaggtggtcagtttcataaagtcattgaatatttccgccttttagggcgtgtgatggccaaagcacttcaagatggacggctattggacgtcccattgagtacagcgttttataaacttattcttggtcaagagcttgatttgcatgatattgtattatttgacgctgaacttggcaagaccttgcaagagctgcgtgttgttgttgcccgcaagcactatctggagggagtaggtggtgacaatagcagcacgatttctgatttatgtttacgtggatgccgaatagaagatctctccttggaattcacgctacctggctatcctgagtacatcctgagatcaggagatgaaattgttgatattactaatcttgaggagtatatatcccttgtcgttgatgctactgtcaagagaggagtcactcggcagatcgaagccttcagatctggattcaatcaggtgtttgacataacatctctacaaatattcaccccttctgagctggactatttgctgtgtggtcgtagagagttgtgggaggtggagactcttgctgaacatatcaaatttgatcatgggtataatgccaaaagtccggcaatcattaacttactggagatcatgggagaacttacagcagatcagcagagggctttctgccaatttgtaactggagctcctaggcttcctcctggtggcttagctgttctgaacccaaagcttacgattgtgagaaagcactcatcgacctcaagtgcagcagccaacggagcaggggcttcggagacagcagatgatgatttgcccagtgtcatgacttgcgcaaactaccttaaactccctccttattctacaaaggaaatcatgtacaagaaactgctctacgccatcaacgaagggcaaggatcgttcgacctctcataa

SEQ ID NO: 2 - protein, 1888 aa, Arabidopsis thaliana
METRSRKRAEATSAAPSSSSSSPPPPPSASGPTTRSKRARLSSSSSSSLAPTPPSSSTTTRSRSSRSAAAAAPMDTSTDSSGFRRGGRGNRGNNNDNSDKGKEKEHDVRIRERERERDRAREQLNMDAAAAAARSADEDDDNDSEDGNGGFMHPNMSSASSALQGLLRKLGAGLDDLLPSSGIGSASSSHLNGRMKKILSGLRAEGEEGKQVEALTQLCEMLSIGTEDSLSTFSVDSFVPVLVGLLNHESNPDIMLLAARALTHLCDVLPSSCAAVVHYGAVSCLVARLLTIEYMDLAEQSLQALKKISQEHPTACLRAGALMAVLSYLDFFSTGVQRVALSTAANMCKKLPSDASDYVMEAVPLLTNLLQYHDSKVLEYASICLTRIAEAFAPYPEKLDELCNHGLVTQAASLISTSNSGGGQASLSVSTYTGLIRLLSTCASGSPLGFRTLLLLGISSILKDILLGSGVSANASVSPALSRPADQIYEIVNLANELLPPLPEGVISLPTSTNALVKGSCQKKSSPSTSGKQEDILKISPREKLLGDQPELLQQFGLDLLPVLVQIYGSSVNGTIRHKCLSVIGKLMYFSSSEMIQSLIGDTNISSFLAGVLAWKDPQVLVPALQVAEILMEKLPETFSKVFVREGVVHAVDQLVLVGKPSHASPTDKDNDCVPGSARSRRYRRRSSNANSDGNQSEEPKNPASLTIGANHNSLDTPTASFMLRETVSSCAKAFKDKYFPSDGGDVDVGVTDDLLHLKNLCTKLTAGIDDHKVKGKGKSKASGPFLGDFSASKEEYLIGVISEILGEISKGDGVSTFEFIGSGVVAALLNYFSCGYFSKEKISELNLPKLRQEGLRRFKAFLEVALPFDGNEGKVPPMTVLIQKLQNALSSLERFPVVLSHPSRSLSGSARLSSGLSALAHPLKLRLCRASGEKTLRDYSSNIVLIDPLASLAAVEEFLWPRVQRSESALKPAAPIGNTEPGTLPSGAGVSSPSSSTPASTTRRHSSRSRSAINIGDTSKKDPVHEKGTSSSKGKGKGVMKPAQADKGPQTRSNAQKRAVLDKDTQMKPASGDSSSEDEELEISPVDIDDALVIEEDDISDDEDDDNEDVLDDSLPMCTPDKVHDVKLADSVDDDGLATSGRQMNPASGGTSGAAAARASDSIDTGIGNSYGSRGALSFAAAAMAGLGAASGRGIRGSRDLHGRTLNRSSDEPSKLIFTAAGKQLSRHLTIYQAVQRQLMLDEDDDDRFGGSDLVSSDGSRFNDIYTIMYQRPDSQVNRLSVGGASSTTPSKSTKSATTNSSVESQSHRASLLDSILQGELPCDLEKSNSTYNVLALLRVLEGLNQLCPRLRAQTLSDRFAEGKITSLDDLSTTAAKVPLDEFVNSKLTPKLARQIQDALALCSGSLPSWCYQLTRACPFLFPFQTRRQYFYSTAFGLSRALNRLQQQQGADGSGSTNEREMRIGRLQRQKVRVSRNRILDSAAKVMEMYSSQKAVLEVEYFGEVGTGLGPTLEFYTLLSHDLQKASLGMWRSSSGDKVSMQIGRDEIEDGKPSAANRDIVLAPLGLFPRPWPSTADISEGGQFHKVIEYFRLLGRVMAKALQDGRLLDVPLSTAFYKLILGQELDLHDIVLFDAELGKTLQELRVVVARKHYLEGVGGDNSSTISDLCLRGCRIEDLSLEFTLPGYPEYILRSGDEIVDITNLEEYISLVVDATVKRGVTRQIEAFRSGFNQVFDITSLQIFTPSELDYLLCGRRELWEVETLAEHIKFDHGYNAKSPAIINLLEIMGELTADQQRAFCQFVTGAPRLPPGGLAVLNPKLTIVRKHSSTSSAAANGAGASETADDDLPSVMTCANYLKLPPYSTKEIMYKKLLYAINEGQGSFDLS

SEQ ID NO: 3 - DNA, 4509 bp, Arabidopsis thaliana
atggagaacagaggccagaaacgaatggaggttgtggaagagttacctgctgataagagagcttgtaactctcaggattttagaccaagcacatccggatcatctgttcaagctcaagctaatgatacgaatccaggacatgaaaacgttgacgctgatatggatacttcttcatctgcttcgccttcgagtcgatcagatgaagaagaacaggaagagcaggataaggaggattcggactatggatcttgcgattctgatgaggaagatccgaggcagagggtgcttcaggattaccagaggcagagatcatctggtgatcatgggaaattgaagtctcttttgttgaatttgactggagaaactgatccttctggacagttatccaggctcactgagttatgtgaagtgttgtcattttctactgaagaatcgctgtccagtgttatggccaacatgctatcaccggtgcttgtaaagttagctaagcatgagaacaatgcagatattatgctcctcgcaattagagctattacttatttgtgtgatgtttatccgccgtcagtagaattccttgtaagacatgataccattcctgctctctgccaaagacttttgactattgagtacttggacgttgctgagcagtgtttgcaagcacttgagaaaatatcccgagatgagccggtagcctgcttgaatgctggagcaattatggcagtgctttcgtttattgatttcttctcaacaagcatacagagagtcgcaatttctactgtggtcaatatatgtaagcagctttcttctgagtctccctcgcctttcatggatgctgttccaatattatgcactcttcttcaatatgaagatcgacagctggtcgagaatgtggctatttgcttgacaaaaatagcagatcaagccagtgagtcaccggcaatgttggatcaactgtgtaggcatggactaattaatgaatcaacacatctcttaaacttgaatagccgcactaccctatctcaacctgtctacaatggtgtgattggaatgctaagaaaactatcttctggttcagctttagctttcagaacgttatatgagcttaacattggctacagtttaaaagaaatcatgtccacgtatgacatttctcattcagtgtcttctacacatcctatcaatgcatgttctaatcaggtgcatgaagtcctgaagttggtgattgagcttcttccagcttcacccgtagaggataatcagctggcatcggaaaaggaaagttttctcgtcaatcagcctgatcttttgcaacaatttggaagagacatgcttcctgtcatgattcaggtgctaaactctggagctaacgtatatgtttcttatggttgcctatcagcaattcacaagctgacttgcttgagtaagtccggtgatattgtcgagttactgaagaacaccaacatgtcaagtgttttggctggcattctgtcaaggaaggatcatcatgtaattgtagtagcactacaggttgcggaagtgcttcttgagaaatacagagatacttttttgaattcttttataaaggaaggtgtttttttcgcgattgaagcactcttaagttctgatagagggcaacaaaatcagggatcagctgacctttcacaaaagcctgttacaaaagagattgtgaaatgcttgtgccaatcttttgaaagatcgctatcctcttcttcacaaacttgtaagattgaaaaggattctgtctacgttcttgcaacacgtatcaaggagggtttctttggacctgaggtattcaactctgagaaaggcttgacagatgtcctccaaaacctcaagaacttgtcggtagcacttagcgagttgatgactgtacccattgatgcgcatgtcctgcatgatgagaaattcttctcaatatggaaccaaatcatggaaaggctgaatggaagggaatctgtgtccacttttgaattcattgagagcggagttgtaaagtcactggcaagttatctttctaatggactctatcaaaggaaacttagcaaagggggtcctgaatgtgatagtttaccatttattggtaagagatttgaggtgttcacaagattgctttggtctgatggagaggcaacttcatccttgttaatacagaagctccaaaattccctttcttctttggaaaacttcccaattgtcctaagccaatttttgaagcagaagaactcatttgcggctattccaaatgggcgttgcactagttatccatgcctaaaagttcgttttctgaaagcagagggggagacttctttgcgtgattactcccaagactttgtcactgttgacccactttgctatttggatgctgtcgatcaatacttgtggcctaaagttaatatagaacctatagattctgtggaagcaaaagatcaagctatagaatgtcaatcttctcaattgcagtcaacttcgatatcttgtcaagctgaaagctcaagtcctatggagattgacagtgagtcttctgatgcgtctcagttgcagggatctcaagtggaagatcagacgcaacttccaggacaacagaatgcttcctcctctgaaacctcctctgaaaaagaggatgcggtacctagacttttgtttcgtctcgaagggcttgaactagaccgttctttgacagtatatcaggcgattctcttgcacaaactaaaatcagaaagtgaagcaaccaacgattcgaagctgagtggaccccacaacatcacttatgaaaggtctgcacaacttggggattctcgtgaaaatctgtttccacctggatctatggaagatgatgagtatcgcccgttcttgtcctatttgtttactcatagacttgctttgcgcctgaaggggtcaagtcatcctccgtatgacatattgtttcttcttaagagtctggagggcatgaacagatttctctttcacctgatttctcttgaacggattaatgcttttggtgaaggtaggctagagaatttggatgatctgagggtacaagttcgtcctgtgccacattctgaatttgttagcagtaagcttacagagaagttagagcagcagcttcgtgattcttttgctgtgtcaacctgcggtctgccaccatggtttaatgatctaatggattcatgtccgtgtttatttagttttgaagccaagtctaaatacttccgacttgcagcctttggttcacagaaaatccgtcatcatccacagcaccttagcagttcaaatgttcatggcgaagcgcgcccagtgactggtagtttacctcgtaaaaagttcttagcttgccgtgaaaacattctagagtctgctgccaaaatgatggagttatatggaaaccagaaggtggtcattgaggttgaatacagtgaagaagtcgggactggtcttgggccaacactggagttctatacgcttgtcagtagggcatttcaaaatcccgatcttggtatgtggagaaatgattgtagttttattgttggaaagccagtcgaacactcgggagttttggcatcttcttcaggactctttccacgcccttggtcaggtacatcaactacgtcagatgtgctgcagaaatttgtcctcttggggacagtggtagcaaaggctttacaagatggacgagtcttagaccttccactttccaaagccttctacaaattaattctcggacaggagttgagttcatttgacatccacttcgttgaccctgaactttgtaaaacactggtggaattgcaagctctggtacgtaggaaaaagcttttcgctgaagcacatggtgattccggagcagccaagtgtgatttaagtttccatggaacaaagattgaggacctttgtcttgaatttgcattgcctggctacacggattatgatctcgctccctattctgcaaatgatatggtaaatttggataacctcgaggaatatatcaagggtattgtcaatgccacagtatgtaatgggatccaaaaacaagtggaagcatttcggtctggatttaatcaggttttctctattgaacatcttcggatattcaacgaagaggagctggaaactatgctgtgtggagaatgtgatctctttagtatgaatgaagtcttggatcacatcaagtttgatcatggatatacttctagcagcccaccagttgaatatttattgcagattctgcatgagtttgatagggagcaacaacgagcctttttgcaatttgtaacaggatctccccggttacctcatggtggtttggcgtctctcagtcccaaactaacaatcgtccgcaagcatggtagcgattcttcagatactgacctccctagtgtgatgacatgcgccaattatctgaagcttcctccttattcatccaaagagaagatgaaggagaagctgatttatgccataacggaaggtcaaggttccttccatctctcttaa

SEQ ID NO: 4 - protein, 1502 aa, Arabidopsis thaliana
MENRGQKRMEVVEELPADKRACNSQDFRPSTSGSSVQAQANDTNPGHENVDADMDTSSSASPSSRSDEEEQEEQDKEDSDYGSCDSDEEDPRQRVLQDYQRQRSSGDHGKLKSLLLNLTGETDPSGQLSRLTELCEVLSFSTEESLSSVMANMLSPVLVKLAKHENNADIMLLAIRAITYLCDVYPPSVEFLVRHDTIPALCQRLLTIEYLDVAEQCLQALEKISRDEPVACLNAGAIMAVLSFIDFFSTSIQRVAISTVVNICKQLSSESPSPFMDAVPILCTLLQYEDRQLVENVAICLTKIADQASESPAMLDQLCRHGLINESTHLLNLNSRTTLSQPVYNGVIGMLRKLSSGSALAFRTLYELNIGYSLKEIMSTYDISHSVSSTHPINACSNQVHEVLKLVIELLPASPVEDNQLASEKESFLVNQPDLLQQFGRDMLPVMIQVLNSGANVYVSYGCLSAIHKLTCLSKSGDIVELLKNTNMSSVLAGILSRKDHHVIVVALQVAEVLLEKYRDTFLNSFIKEGVFFAIEALLSSDRGQQNQGSADLSQKPVTKEIVKCLCQSFERSLSSSSQTCKIEKDSVYVLATRIKEGFFGPEVFNSEKGLTDVLQNLKNLSVALSELMTVPIDAHVLHDEKFFSIWNQIMERLNGRESVSTFEFIESGVVKSLASYLSNGLYQRKLSKGGPECDSLPFIGKRFEVFTRLLWSDGEATSSLLIQKLQNSLSSLENFPIVLSQFLKQKNSFAAIPNGRCTSYPCLKVRFLKAEGETSLRDYSQDFVTVDPLCYLDAVDQYLWPKVNIEPIDSVEAKDQAIECQSSQLQSTSISCQAESSSPMEIDSESSDASQLQGSQVEDQTQLPGQQNASSSETSSEKEDAVPRLLFRLEGLELDRSLTVYQAILLHKLKSESEATNDSKLSGPHNITYERSAQLGDSRENLFPPGSMEDDEYRPFLSYLFTHRLALRLKGSSHPPYDILFLLKSLEGMNRFLFHLISLERINAFGEGRLENLDDLRVQVRPVPHSEFVSSKLTEKLEQQLRDSFAVSTCGLPPWFNDLMDSCPCLFSFEAKSKYFRLAAFGSQKIRHHPQHLSSSNVHGEARPVTGSLPRKKFLACRENILESAAKMMELYGNQKVVIEVEYSEEVGTGLGPTLEFYTLVSRAFQNPDLGMWRNDCSFIVGKPVEHSGVLASSSGLFPRPWSGTSTTSDVLQKFVLLGTVVAKALQDGRVLDLPLSKAFYKLILGQELSSFDIHFVDPELCKTLVELQALVRRKKLFAEAHGDSGAAKCDLSFHGTKIEDLCLEFALPGYTDYDLAPYSANDMVNLDNLEEYIKGIVNATVCNGIQKQVEAFRSGFNQVFSIEHLRIFNEEELETMLCGECDLFSMNEVLDHIKFDHGYTSSSPPVEYLLQILHEFDREQQRAFLQFVTGSPRLPHGGLASLSPKLTIVRKHGSDSSDTDLPSVMTCANYLKLPPYSSKEKMKEKLIYAITEGQGSFHLS

SEQ ID NO: 5 - DNA, 4737 bp, Solanum lycopersicum
atgggaaaccgggggcagaaaaggactgaaaatgttgatgaactgcctgccgataagcgaccctgtagctcaaccaatgacaggcctagtacttccaactcagtgattcctactacaatgagttccatacacgaaagtcaccatggtgatatagacacatcttcatcatcatcatccacttcagggtcaagtgaaggtgaaaaggactctgcttatggatcttatgaatctgataatacttatagggactattacaggcagcaattgatgggcaatcagagcaaattcaatggagttttggaaagtttgagaaaagaatctgaagaatcagcactgctggctgctcttacggaactatgtgatttgttatcgttttctcctgatagttcgatgtcgaacgtaatggcagatttattttctcccgttcttgttagattggctagatatgagagcaattctgaaataatgctattagcaatcagggcaatgacttatttatgtgaagttcatccccgttcgtcggcctcgcttgccaatcatgacgcagttcctgccctttgccaaagactaatggccattgagtttttggatgtggctgaacagtgtttgcaagcactagagaaaatctcgcgggagcaacctatagtgtgtttgcagtctggggctataatggccattttacgttacattgatttcttttcgacaagtgagcagaggaaggcactgttgacagtcgtaaatatttgtaaaaagcttccctccggatgtcctccacctttaatggaggcggttcccgttttgtgcgatcttcttctatatgaggatagacagcttgttgagagcgtagcaacttgtttgattagaatagtcgagcaggcatcccattcttcagagatgctggaccaactgtgtaatcacaggctagttcagcaagtcactcatctcatagagttgaatggaagaacaacagttagccaatcagtttatgttggtttaattgggttacttgtcaaactggctgctggctctattgttgctgtcaagactctctttgaacgtaacatcagccacatattaaaggacattttatccactcatgacttctcacatggggtgccttctactctgattgttgatgggcattataatcaggtagatgaagttctcaagttgttaaatcaacttcttcctcccatatccagagagcagaatatcaaactagcagcagacaaggaagatttcctcgtcaacaatccggatcttctggaggaatttggatttcatttacttcctgtgctgatccaggtggttattcttatttgtggttatataaattaccttgctctagcttcccctgactcttctttaatcgttaaacaggtggtcaattctggcatgagtttaaatgcattgtttggctgtctctctgtcatcaataagttggtttatttcagcaaatttgacaggcttgaatttcttcaaaatactaacatttcaagcttcttagcaggagtttttactcgcagagatcctcatgttctgatattagcccttcaaattgttgataagctattagagaagctctctcatattttcttggactcatttgttaaggaaggtgttctttttgctgttgatgcacttctttccctgcaaaaatgttcgcagtctctgttttcgaccaatggtgttcaagcatcagatgaaaccagccaaggatcagcaccacctactgcagtaaattgtctttgttttgcttctgatgctcttaagtctccaacaggaccagaatcaaggacttgcaagatagagaaagagactgtccaaagtcttgctaggcatataaagaccaattactttgcaacagactcaatgaactccagattaggaataaccgatgttcttcagaagctcaagactctttcgtctcagttaactgatctggttcacaaatttagtagcagcattgctcctcctcaagagaaagaagacttttaccctgttttgcatcaaattatgtcagagttaaatggaaataatgccatttctacgttcgagttcattgagagtggagttgttaagtctctagtaaattacctctccaatggccaatacttgggaaaaaaggtagatggtgatgtctcagtaaatcagctgtatattatagaaaagagatttgagctgtttggtagattacttttggataactctggcccgcttgtggagaactccacttttctagctttgataaggagattgcatagtgcactttgctctgttgagaacttcccagtcatcttgagtcatgcatctaagctacgaaactcatatgctacaatcccatatgagcattgtacgccatatccttgtctgaaggtccagtttgtgaagggagagggggagtcatcacttgttgattatccggagagtgttgtgagcgtagatcccttttcgctgttggaaacaattgagggatacctgtggccaaaagtgagtaaaaagaaaagtgaaaagttgaatccacccactctggatttggaggaagagtcaccatctcgtgcatcacaagatgtaagcacgtctcaaggtaaaaatccaggacccatggaatcggacaccacttcaacagattctcatgaaacacaggttgtgaagaataacttgcaattatttgctgaagtggaaactgtggatgtagaacaaacaaagagtgtcccaatggatatttcagatgttaatgcagagttattgaagaaaggaagactgaattcatctgaagatgatagtagtacaagtttggaatgtactggatgttgtgatgatgaaaatgttgcacctaaattgatattctacctggagggacagaagttgaaccacaagttgaccctatatcaaactctactcctgcggcagattaaagcagagaatgacatcactactaattcaagcgtgtggagtcaagtacacagggtgacctacagaaaatttgtgagacataaaccaggatgtcctcacagttgcaaacatgctgtacattctacatcatctgagaaatctacagcatggtggcagttcaccccatctttctctagcatgttcggttctgaaatggttgatcttgagaaatcaagtccaacttatgatatcttatttcttcttagaagcttggaaggtttgaacaggttcagtattcatcttgggtctcgaacaaaactatatgcttttgctgaaggaaagactaccaattttggtgatcttaaggttacaaattctgatctccctcagaatgaatttgcaagcactaaattgacagaaaaaatagaactgcaaatgaggagtcccttttctgtttccataggtggtttgccaccttggtgtgaacaattggttaatacatgcccctttttgtttggtttcgaagcaagatgcaagtatttccgccttgctgcatttggtcgacagccaattcagcctgaatcatcgtctcataatacagctacaggtgtgagtggtaggcaccaaaacagtagtgttttacgccggaaaaaattcttagttcatcgaagtagaattttggattctgctaggcagatgatggacctccatgccaatcagaaggttgtcattgaggtggaatataatgatgaggttggtactggtcttggtccgacgctagaatttttcacctttgtcagtcatgagttccagaagattgggctagggatgtggagaggtgattacttggctcatgccagcatgagtgtagaggaggaatctggaattattttctctccttttggtctgttcccccgcccatggtcaccttcaccccattcattaaatggcctagagttctctgaagtgctgaaaaagtttgtgcttctgggccagatagttgcaaagtctcttcaagatggcagggttctagatcttcggttatccagagcattttacaagcttcttcttgggaaggaactcactgtgtatgacatccagtcatttgaccctgaacttggtggagttctcctagaatttcaggctcttgttgaaagaaaaagacatctggaatcacatcctgagggaaaatcatcgttagacctagaacttaatttccggaatacaaaaattggtgatctttgtcttgactatactcttcctggctatccagattatgtccttagttctgcatctgatgcaaaaacggttgactcctctaacttagaggaatatgttttacttgttgtggatgctactctgaattctggaattttaagacaaattggagcattcaagtcgggctttgatcaggttttccccatcagacatcttcaggttttcactgaagatgaattagagagactattgtgcggagagtgtggattctggaactccaatgagcttctggatcacatcaagtttgaccatgggtacactgccaacagtcctccagttttaaatttacttgaaattatgaaggaatttgacagcaagcaacagagagcattcctgcagtttgtcactggtgcacctagactgcctccagggggtctggcatctcttagcccaaagttaacaatcgttcggaagagttgcagtgtttgggtcgacgctgacctacctagtgtgatgacatgtgcaaattatctcaagctaccaccatactcttcaaaagagaaaatgaaggaaaagctgttatatgccataacggaaggacaaggctcattccatctttcatag

SEQ ID NO: 6 - protein, 1578 aa, Solanum lycopersicum
MGNRGQKRTENVDELPADKRPCSSTNDRPSTSNSVIPTTMSSIHESHHGDIDTSSSSSSTSGSSEGEKDSAYGSYESDNTYRDYYRQQLMGNQSKFNGVLESLRKESEESALLAALTELCDLLSFSPDSSMSNVMADLFSPVLVRLARYESNSEIMLLAIRAMTYLCEVHPRSSASLANHDAVPALCQRLMAIEFLDVAEQCLQALEKISREQPIVCLQSGAIMAILRYIDFFSTSEQRKALLTVVNICKKLPSGCPPPLMEAVPVLCDLLLYEDRQLVESVATCLIRIVEQASHSSEMLDQLCNHRLVQQVTHLIELNGRTTVSQSVYVGLIGLLVKLAAGSIVAVKTLFERNISHILKDILSTHDFSHGVPSTLIVDGHYNQVDEVLKLLNQLLPPISREQNIKLAADKEDFLVNNPDLLEEFGFHLLPVLIQVVILICGYINYLALASPDSSLIVKQVVNSGMSLNALFGCLSVINKLVYFSKFDRLEFLQNTNISSFLAGVFTRRDPHVLILALQIVDKLLEKLSHIFLDSFVKEGVLFAVDALLSLQKCSQSLFSTNGVQASDETSQGSAPPTAVNCLCFASDALKSPTGPESRTCKIEKETVQSLARHIKTNYFATDSMNSRLGITDVLQKLKTLSSQLTDLVHKFSSSIAPPQEKEDFYPVLHQIMSELNGNNAISTFEFIESGVVKSLVNYLSNGQYLGKKVDGDVSVNQLYIIEKRFELFGRLLLDNSGPLVENSTFLALIRRLHSALCSVENFPVILSHASKLRNSYATIPYEHCTPYPCLKVQFVKGEGESSLVDYPESVVSVDPFSLLETIEGYLWPKVSKKKSEKLNPPTLDLEEESPSRASQDVSTSQGKNPGPMESDTTSTDSHETQVVKNNLQLFAEVETVDVEQTKSVPMDISDVNAELLKKGRLNSSEDDSSTSLECTGCCDDENVAPKLIFYLEGQKLNHKLTLYQTLLLRQIKAENDITTNSSVWSQVHRVTYRKFVRHKPGCPHSCKHAVHSTSSEKSTAWWQFTPSFSSMFGSEMVDLEKSSPTYDILFLLRSLEGLNRFSIHLGSRTKLYAFAEGKTTNFGDLKVTNSDLPQNEFASTKLTEKIELQMRSPFSVSIGGLPPWCEQLVNTCPFLFGFEARCKYFRLAAFGRQPIQPESSSHNTATGVSGRHQNSSVLRRKKFLVHRSRILDSARQMMDLHANQKVVIEVEYNDEVGTGLGPTLEFFTFVSHEFQKIGLGMWRGDYLAHASMSVEEESGIIFSPFGLFPRPWSPSPHSLNGLEFSEVLKKFVLLGQIVAKSLQDGRVLDLRLSRAFYKLLLGKELTVYDIQSFDPELGGVLLEFQALVERKRHLESHPEGKSSLDLELNFRNTKIGDLCLDYTLPGYPDYVLSSASDAKTVDSSNLEEYVLLVVDATLNSGILRQIGAFKSGFDQVFPIRHLQVFTEDELERLLCGECGFWNSNELLDHIKFDHGYTANSPPVLNLLEIMKEFDSKQQRAFLQFVTGAPRLPPGGLASLSPKLTIVRKSCSVWVDADLPSVMTCANYLKLPPYSSKEKMKEKLLYAITEGQGSFHLS

SEQ ID NO: 7 - DNA, 5553 bp, Solanum lycopersicum
atggaaactcggagccggaaacgaacggaggccacgtcatcagcgccttctgcttcttctccttcatcaggtcccaccacacgcgctgttaagaaagctcgttttaccacacgcgccgcctcaaactcgatctcaactcgttcccgactcacaaatcgttcccaagacctacaatcgatggactccacgaatgaatcatccgggtctggcagccgaaccaggcggggaaagaatcacgggttagatagaaataatccggagaagggtaaggagaaagagcacgaaattagggatagagacagagatatgggattgaacatggatactgatgggggtgatgaagatgataatgaaagtgaaggtggtgctgggattttgcaacataatttgacttcagcaagtagtgcacttcaaggactgttgagaaaattgggtgctggtttggatgatttactgccgagttcagcaatggtgtccgcttcctcgtcgcaacagaatgggcgtctgaagaagatattatcgggcttgagagctgacggggaagaagggaagcaaatagaggcattgacgcagctttgtgtgatgctttccattgggacagaagactctttgagcactttttcagtggactcttttgtacctgtcctggtggggctgcttaatcatatgagtaatcctgatattatgcttctcgcagctagggcgttaacccatttggttgatgttctgccatcttcttgtgctgctgttgtgcattatggagcggtttcatgttttgtagctcgcttactcacaattgaatacatggacttagctgagcagtctctacaagctttaaagaagatatctcaagaagatccaactgcttgtttgcaagcaggtgcactcatggctgtgctgtcgtatctcgatttcttttccactggtgttcagagagtagcactagcaactgctgctaatatgtgcaagaagctgccttcggatgctgctgactttgtgatggaagctgttccattgttgacgaatctccttcagtatcatgatgcaaaggtattagagcatgcttctatctgcttgacccggatagctgaagcatttgcatcatctccagaaaagctagatgaactctgtaatcacggacttgtcacacaggctgcctccctcatctcaaccagtaattctggaggtggtcaggcttcactcagcacggaaacttacacaggcttgatccggcttctttgtacttgtgccagtggctcaccattaggggctaaaaccttgatgatgcttggtatcagtgggatcctcaaggacattttatcagcctctgtctctatttcacctgccatgagcagacctgcggagcagatttttgagattgtgaatcttgcaaatgaactacttcctccgctgcctcaaggaattatctctcttcctgttagcacaaatttgttcattagaggtccttttacgcggaaatcctctgctagtggttctagcaaacaggaggatcttaatgcatcttctcaggaggtatcagctcatgagaaactattgaatgatcaacctgaacttctgcaacaatttggaatggatctccttcctgttctgatacagacatatggatccagtgtaaatacagcagcacgccacaaatgcctctcagttattggaaaacttatgtatttcagtaatgcagatatgattcaatctttaactaatgacactaacttgtcaagtttcttggctggggttttggcgtggaaggatccccaagtattggtccccgctcttcaaatagcagagattctaatggagaagctccctggagtttttggcaagatgtttgtccgggaaggtgttgttcatgctgtagatgccttgatgttgtctgggtctcatgtttctgctcctccccatccaacacgtgctgagaaagagaaacataatagacgccgtagcactaattccaatacagatgcaatttctgttgaagatcttacaagtccagttccaagtactggatctctgccaaattcaatggaaattcggaccgttaattctagcctccggatgtcagtcagtacatgtgcaaaagctttcaaggataaatacttcccatcagattctgaggctgctgaagctggtgtcacggatgatcttatacgattgaagaatctctgcatgaagttgaatgctggtattgatgagcagatagctaaacctaaaggaaaatccaaaacatttggtcctcagcttggggatagctatgttggaaaagaagaaaacttggctgaagtgatagctgccatgatgggggaactcagcaaaggggatggtgtttcaacttttgagttcagtggaagtggagttgttgcttctttgctgaaatattttacgtttgcgtacttttctaaggaaagaatctctgatactagtatgtctaagcttcgacaacaagcaatcagaagatacaagtcttttattgcagttgcccttcctgctggtgttgatggtggaaatatggttcccatgactgttctggtccaaaagcttcaaaatgctctatgttcattggagcgttttcctgttgtattgagtcatagttccagatcatcgacaggaaatgcacgtctttcttcaggtttaagtgttttgtctcagccttttaagctgcgcctttgcagagctcaaggagagaaaaccctccgtgactactcttcaaatgttttgctgattgatcctttggcaagtttagtagctattgaagaattcctttgggcccgagttgggagacctgaggctgaacagaaggcatctgctactggtggaaactctgggtctgggactatacctgctggaggcagtgcgtcatctccatctatgtccactcctgcctctgcatctcgtcgtcattctgctcgatcaaggtcagcagttaatattaatgaaagtgatggaagctcttcaaagggcaaaggtaaagcggttttgaagcctgctcaaaaagatcgcaggggaattcgatcaagagatcctgttaaaataagagctgccttggagaaggccttaagagaggagcctgttgatggggagactagttcagaggatgacgagctgcatccttctctcattgaacttgatgatgctttggtgattgaggatgatatgttcgatgaagatgaagatgaccatgatgatgtgctgagggatgatccttttcctgtctgcatggcagatgaagtgcatgatgttaaattgggagactcttcggaggatagcccttttgcacagacaccaactggcagcaatacaaatgctggtggtggttctgggagcagaattgcttctgctcggggatctgattccgttgagttcagaagtaggaactcgtatggttcaaggggggcaatgtcatttgctgctgctgccatggctggtctttcatctgctagtgttagaggtgtgaggggcgctagagatcgacatgggcatcctctactcagctctggtgatccaccaaaactaatattttctgttggtgggaagccgcttaataggcagttgactatctaccaggctatccagcggcagcttgttctagacgaggatgatgatgagagatatggtggcaatgattttgtatctggtgacggcagtagggtttggagtgatatttacacgatcacataccagagggcagacaaccaagctgagaggtcaagtgggtctgggagttcaatttccaagtctatgaaaaccagttcttcaacaagttccggtgctgatccttcattggttcaagcatcattgttagatagtatattgcagggagaacttccttgtgatctggagaaaagtaaccctacttacagtattttgtacctcttacgtgtattggaggcgctgaatcagcttgccccccgtttgagagtcctgtccatgattgatgatttctctgaaggaaaaatttctagtctagatgagctcggtactacgggtatcaaaatcccttctgaggaatttgtcaatagtaagctcactccgaaattggcacgacagatccaggatgctcttgcactttgtagtggatctcttccatcttggtgttaccagttgaccaaggcctgcccatttctttttccatttgagactcggcgccagtacttctattcaactgcttttgggttgtcacgtgctttatataggctgcagcaacagcaaggtgctgatggtaatgggtctactcatgagagagcagttagggttggcagattacagcgccagaaagttcgtgtctcaaggaaccgcattctggattctgctgcaaaagtaatggagatgtactctagccaaaaagctgttcttgaagttgaatattttggtgaagttggtactggcctgggtcctacacttgagttttatacccttataagtcacgatctacagaaacttggacttggaatgtggagatctggtttatcattaacttcaaatgaacattctgtggaagttcatatcgataataaattaagtagaagtgacggagatcttgtccaagcacctcttggattattcccacgtccctggtcaccacatactggtactgttgatggaggtcaattctataaagcaattgaatatttccgcttgcttggacgtgttatggcgaaagctcttcaagatggacggcttttggaccttccactgtccatggccttctataagctcgttcttggtcaagaacttgatttgtatgatattctttcttttgacaccgaattggggaagactttgcaagagttgcaagccctcgtcagtcgaaagcaatatatagaatcaataaaagatcagaacctggacgagtcttatgacatgcattttcgtgggactccagttgaggatctttgtttagatttcacacttcctggctatcctgaatatattcttaaagcaggcgacgagaatgtgagtcgcgatatcgtggattttaacttggaggagtatatttctttggtagttgatgctactgtgaaaactggaatcaggcagcaaatggaggcttttagatctggcttcaatcaggttttcgacttttcagctctgcaaatattctctccttcagagttagactatctattatgtggccgtagagagctgtggaagcctgagacgctagtagatcacataaaattcgatcatggattcacatccaagagtcctcctattattcatttactagagattatgggagagttcacacctgagcagcaacgagcattctgccagtttgttactggtgctcctcggctccccgcaggtggtcttgcttctctgaatcctaagttgacaattgtgaggaagcattcatctagtgctggcaatgcagcacagaacagtaatgccccatcagaatctgcagatgaagacctacccagtgtgatgacatgtgctaattacttgaaactccctccctattctactaaggagatcatgtccaagaaattactctatgccattaatgaaggtcaaggatcgtttgatttgtcataa

SEQ ID NO: 8 - protein, 1850 aa, Solanum lycopersicum
METRSRKRTEATSSAPSASSPSSGPTTRAVKKARFTTRAASNSISTRSRLTNRSQDLQSMDSTNESSGSGSRTRRGKNHGLDRNNPEKGKEKEHEIRDRDRDMGLNMDTDGGDEDDNESEGGAGILQHNLTSASSALQGLLRKLGAGLDDLLPSSAMVSASSSQQNGRLKKILSGLRADGEEGKQIEALTQLCVMLSIGTEDSLSTFSVDSFVPVLVGLLNHMSNPDIMLLAARALTHLVDVLPSSCAAVVHYGAVSCFVARLLTIEYMDLAEQSLQALKKISQEDPTACLQAGALMAVLSYLDFFSTGVQRVALATAANMCKKLPSDAADFVMEAVPLLTNLLQYHDAKVLEHASICLTRIAEAFASSPEKLDELCNHGLVTQAASLISTSNSGGGQASLSTETYTGLIRLLCTCASGSPLGAKTLMMLGISGILKDILSASVSISPAMSRPAEQIFEIVNLANELLPPLPQGIISLPVSTNLFIRGPFTRKSSASGSSKQEDLNASSQEVSAHEKLLNDQPELLQQFGMDLLPVLIQTYGSSVNTAARHKCLSVIGKLMYFSNADMIQSLTNDTNLSSFLAGVLAWKDPQVLVPALQIAEILMEKLPGVFGKMFVREGVVHAVDALMLSGSHVSAPPHPTRAEKEKHNRRRSTNSNTDAISVEDLTSPVPSTGSLPNSMEIRTVNSSLRMSVSTCAKAFKDKYFPSDSEAAEAGVTDDLIRLKNLCMKLNAGIDEQIAKPKGKSKTFGPQLGDSYVGKEENLAEVIAAMMGELSKGDGVSTFEFSGSGVVASLLKYFTFAYFSKERISDTSMSKLRQQAIRRYKSFIAVALPAGVDGGNMVPMTVLVQKLQNALCSLERFPVVLSHSSRSSTGNARLSSGLSVLSQPFKLRLCRAQGEKTLRDYSSNVLLIDPLASLVAIEEFLWARVGRPEAEQKASATGGNSGSGTIPAGGSASSPSMSTPASASRRHSARSRSAVNINESDGSSSKGKGKAVLKPAQKDRRGIRSRDPVKIRAALEKALREEPVDGETSSEDDELHPSLIELDDALVIEDDMFDEDEDDHDDVLRDDPFPVCMADEVHDVKLGDSSEDSPFAQTPTGSNTNAGGGSGSRIASARGSDSVEFRSRNSYGSRGAMSFAAAAMAGLSSASVRGVRGARDRHGHPLLSSGDPPKLIFSVGGKPLNRQLTIYQAIQRQLVLDEDDDERYGGNDFVSGDGSRVWSDIYTITYQRADNQAERSSGSGSSISKSMKTSSSTSSGADPSLVQASLLDSILQGELPCDLEKSNPTYSILYLLRVLEALNQLAPRLRVLSMIDDFSEGKISSLDELGTTGIKIPSEEFVNSKLTPKLARQIQDALALCSGSLPSWCYQLTKACPFLFPFETRRQYFYSTAFGLSRALYRLQQQQGADGNGSTHERAVRVGRLQRQKVRVSRNRILDSAAKVMEMYSSQKAVLEVEYFGEVGTGLGPTLEFYTLISHDLQKLGLGMWRSGLSLTSNEHSVEVHIDNKLSRSDGDLVQAPLGLFPRPWSPHTGTVDGGQFYKAIEYFRLLGRVMAKALQDGRLLDLPLSMAFYKLVLGQELDLYDILSFDTELGKTLQELQALVSRKQYIESIKDQNLDESYDMHFRGTPVEDLCLDFTLPGYPEYILKAGDENVSRDIVDFNLEEYISLVVDATVKTGIRQQMEAFRSGFNQVFDFSALQIFSPSELDYLLCGRRELWKPETLVDHIKFDHGFTSKSPPIIHLLEIMGEFTPEQQRAFCQFVTGAPRLPAGGLASLNPKLTIVRKHSSSAGNAAQNSNAPSESADEDLPSVMTCANYLKLPPYSTKEIMSKKLLYAINEGQGSFDLS

SEQ ID NO: 9 - DNA, 3612 bp, Oryza sativa
atggagtgccccaaggagtgcctcagccacggcgtgccagccgccgtgctgcagttcttcgacttcttctcgatgcacaagcagaagctggtgctcaagatcgtcgccaacgtcttgggcgacttcagcgcgaaggatgcggccaaggccatggaggccgcgcccgttctgtgcaacctcctgcaatccactgacaagacgatactcgactccgccgtttcttgcttggttttggtctctgatggtgcttgcgacagtgcccaacacatggaaaagctttacgagcttaatgcagtccaagcgacgatgaggttgatggagaacgacgggtggaagagcctcagcgatgagactttatctggcatccttggtcttctcaaagacctagcttctctctcagcaagggctgtaaagtctctttttgagttaaacatttgtgatttgctcaagcagatgataacatactacacctcgtcgcacagtgatcacaataaggtgcagacgcttgtagagctcatttattatcttatgccacctcttgaaatgtgtgaccatcgtaccgaactaatcattgcaaagaagaatgtcatcacagaacaaagtggatacatccaacagcttgctagcatccttacttttataatacaggttgcgaaatctgctgcactatcatcaatttgctacagttgtgttgttgtcatcagaaacattgttgaattaagcacaccttcttccttggtggaggtacagaagacagtaaacctgtcaagcttacttgctggctggttggcccggaagaaccgccatatcatattccaaacgctcaacgtttcgaagacccttctgagaaaagaccagaaattcttctttgagaccttcatcagggagggtctaaagcatgcaattgatgcaatactaacacaggaaaaaggaaagagccgcttgccagaaagttgcctttgttttgatttagacttggagacctcgacagatgatgcatgcaggattaataatggtgctatcctgaaactagcggaggagataaagaaaaacttcttggtaaaggttgccaagtctcctcacaagtttgggtgtgcttttaaaagcataaaggaatttttttctcgtttgaattgtcatgccacggcacccccagctaaagatcaggatctctgcaagcagttgtctgatttttcaaggcaattattatcggatgaactgccaagtacttctacttttgagtttgtgcagagtggatctatcaaacatttggcaggttatctttccaatgggacatactttaattcaaatctcaggaattgccaggacttgataggggagcttaaggaggtgaaaatccggctgcagaagttcacgcacttggctctcagcgtggacaatgaaagctcggtgaagccacttgagattttggtggagaaactgatagatgcgttgcatgtgtggtatgacagtttccctgtaatcctggctgatgaacagtgcacacgtgagagcaccatgattcctctgagggattcaggaactgaggaaccaatgtcactatatataaaattttcgagatcagccagggaggaggagttggaggattatggtggagttctccctgttgatctttcttcgacacctgaatccattgaagaggtcctgttgcctgagatctgtaaaagaactggcaatgaaacttcatacaaggaaaacactcaagaagcaaatgggagcagaaaatctgttgggctcagaaatggtgacgggcacaagttctcaagattgaaattctcttacaaaggaacacaactccagtcatctacaccactttttgagtcaatcctccgctcaatgcatgaaggagaaaccgatctccagattgacccatctttttgggataaagaacacaagatagtatacagaagaagaaacaaaagcaagaaaatatcttcccatagttcctacaatattcagttgtgccgtgtgcatgaaaaacttgaaatgtcattgcttaaggacccctttttctccaccatactcactggcaagcttcctggtgatctggatgaatctgatccatcatataacttcctgttcatgctgaaagtcctcgaagggctcaaccgtttttcatatcatctatcaatggatgataagttatgcaaatttgctgaaggctgcctccaagagtttgatgaccttaaggtggcaatttgtccaattccacgggatcagttcgtgagcagtctactgacaaataagttagagcagcaaatgcaagatagcttgtttggggatggcttgataccctcgtggtgtatctatttggttgaaacttgcccgttcttgttgtcattcgaagctcgatggaagtatttctgcctgacggcacatcactcattcatgacagatgaggctagcagttcaacagaaactaagaagtacagcgtaacacggagcaaaatccttgaagatgcttcatcgatgttgaacaaacatggatcagacaccaaattcattgaggtggaatttgatggagaggttgggaccggtcgaggcccaaccttcgaattctataccacagttagtcatgaactacagagagtgggtcttggaatgtggagaggagacgacaccagccaagaatgcgaagctggttttgtccatgccccttttggtctctttccacagccatggtcctcagcaaacacttcatctcaagggatcagtttgtccaatgtggtacaaaaattcaagcttcttgggcatcttgtagcaagagcagttttggatggaagggttctggatattcctctctcgaaagcattttacaagatcatgcttgagcaggaccttgatatttatgacattccatcatttgatcccaagttgggcaagactgttatggagtttcaagcacttgttaaaaggaagaagttcctggaggaaagggcatccaatccagcagctgatttgtcctataaaaacgtgcgattggaggatttatgtcttgactttacccttcctggaaatccggaatatgaacttgtccctggaggttcagagaagatggtgacacttgacaatttggaggagtatgtgtcttcaattgttgatgcaaccttgaaaagtgggatatccaatcaaatagaagctttcaaggctggaattaacaaggtttttgctcttaagactcttcggttgttcagtgaggatgagatggagcgtatactatgtggcgaacaagattcttgggcttcgaacaaacttgaggatcacatcaattttgattatggatatgatgcgaacagtgcatcagtaattagtttcctggagatcttgcgggagtttggaagagaggaccagcgggcgttcttgcattttacgactggagctcctcagctcccacttggtggcctagcttcgctcgatcctaagctcaccgtagtgcgaaagcaatgtgatggcaaagtagacaacgaattaccgagtgtcaatacttgccggcatttcttcaagcttccaccgtactcctctaaggagattatgagacagaagctcaaatatgctatcaaggagggtttaggctccttccaattatcatga

SEQ ID NO: 10 - protein, 1203 aa, Oryza sativa
MECPKECLSHGVPAAVLQFFDFFSMHKQKLVLKIVANVLGDFSAKDAAKAMEAAPVLCNLLQSTDKTILDSAVSCLVLVSDGACDSAQHMEKLYELNAVQATMRLMENDGWKSLSDETLSGILGLLKDLASLSARAVKSLFELNICDLLKQMITYYTSSHSDHNKVQTLVELIYYLMPPLEMCDHRTELIIAKKNVITEQSGYIQQLASILTFIIQVAKSAALSSICYSCVVVIRNIVELSTPSSLVEVQKTVNLSSLLAGWLARKNRHIIFQTLNVSKTLLRKDQKFFFETFIREGLKHAIDAILTQEKGKSRLPESCLCFDLDLETSTDDACRINNGAILKLAEEIKKNFLVKVAKSPHKFGCAFKSIKEFFSRLNCHATAPPAKDQDLCKQLSDFSRQLLSDELPSTSTFEFVQSGSIKHLAGYLSNGTYFNSNLRNCQDLIGELKEVKIRLQKFTHLALSVDNESSVKPLEILVEKLIDALHVWYDSFPVILADEQCTRESTMIPLRDSGTEEPMSLYIKFSRSAREEELEDYGGVLPVDLSSTPESIEEVLLPEICKRTGNETSYKENTQEANGSRKSVGLRNGDGHKFSRLKFSYKGTQLQSSTPLFESILRSMHEGETDLQIDPSFWDKEHKIVYRRRNKSKKISSHSSYNIQLCRVHEKLEMSLLKDPFFSTILTGKLPGDLDESDPSYNFLFMLKVLEGLNRFSYHLSMDDKLCKFAEGCLQEFDDLKVAICPIPRDQFVSSLLTNKLEQQMQDSLFGDGLIPSWCIYLVETCPFLLSFEARWKYFCLTAHHSFMTDEASSSTETKKYSVTRSKILEDASSMLNKHGSDTKFIEVEFDGEVGTGRGPTFEFYTTVSHELQRVGLGMWRGDDTSQECEAGFVHAPFGLFPQPWSSANTSSQGISLSNVVQKFKLLGHLVARAVLDGRVLDIPLSKAFYKIMLEQDLDIYDIPSFDPKLGKTVMEFQALVKRKKFLEERASNPAADLSYKNVRLEDLCLDFTLPGNPEYELVPGGSEKMVTLDNLEEYVSSIVDATLKSGISNQIEAFKAGINKVFALKTLRLFSEDEMERILCGEQDSWASNKLEDHINFDYGYDANSASVISFLEILREFGREDQRAFLHFTTGAPQLPLGGLASLDPKLTVVRKQCDGKVDNELPSVNTCRHFFKLPPYSSKEIMRQKLKYAIKEGLGSFQLS